European Patent Specification EP 3 585 443 B1, published May 7, 2025. Title: REGULATION OF GENE EXPRESSION BY APTAMER-MEDIATED ACCESSIBILITY OF POLYADENYLATION SIGNALS. Applicant: MeiraGTx UK II Limited Guo, Xuecui Han, Joonhee Zhong, Zhaojing. The sequence listing filed with the application follows.

SEQUENCE LISTING (17 sequences)

SEQ ID NO: 1 - DNA, 332 bp, Artificial Sequence
  Synthetic construct
aaggccaagaagggcggaaagatcgccgtgtaagccataccacatttgtagaggttttacttgctttaaaaaacctcccacacctccccctgaacctgaaacataaaatgaatgcaattgttgttgttaacttgtttattgcagcttataatggttacaaataaagcaatagcatcacaaatttctaaaggtataatcgcgtggatatggcacgcaagtttctaccgggcaccgtaaatgtccgactacctttatttcgaaagaaataaagcatttttttcactgcattctagttgtggtttgtccaaactcatcaatgtatcttaacgcgt

SEQ ID NO: 2 - DNA, 333 bp, Artificial Sequence
  Synthetic Construct
aaggccaagaagggcggaaagatcgccgtgtaagccataccacatttgtagaggttttacttgctttaaaaaacctcccacacctccccctgaacctgaaacataaaatgaatgcaattgttgttgttaacttgtttattgcagcttataatggttacaaataaagcaatagcatcacaaatttcacataaagcataatcgcgtggatatggcacgcaagtttctaccgggcaccgtaaatgtccgactgctttatttcgaaagaaataaagcatttttttcactgcattctagttgtggtttgtccaaactcatcaatgtatcttaacgcgt

SEQ ID NO: 3 - DNA, 335 bp, Artificial Sequence
  Synthetic construct
aaggccaagaagggcggaaagatcgccgtgtaagccataccacatttgtagaggttttacttgctttaaaaaacctcccacacctccccctgaacctgaaacataaaatgaatgcaattgttgttgttaacttgtttattgcagcttataatggttacaaataaagcaatagcatcacaaatttaataaagataatcgcgtggatatggcacgcaagtttctaccgggcaccgtaaatgtccgactctttatttgtgcgaaagcacaaataaagcatttttttcactgcattctagttgtggtttgtccaaactcatcaatgtatcttaacgcgt

SEQ ID NO: 4 - DNA, 337 bp, Artificial Sequence
  Synthetic construct
aaggccaagaagggcggaaagatcgccgtgtaagccataccacatttgtagaggttttacttgctttaaaaaacctcccacacctccccctgaacctgaaacataaaatgaatgcaattgttgttgttaacttgtttattgcagcttataatggttacaaataaagcaatagcatcacaaattttaaagcaataatcgcgtggatatggcacgcaagtttctaccgggcaccgtaaatgtccgacttgctttatttgtgcgaaagcacaaataaagcatttttttcactgcattctagttgtggtttgtccaaactcatcaatgtatcttaacgcgt

SEQ ID NO: 5 - DNA, 331 bp, Artificial Sequence
  Synthetic construct
aaggccaagaagggcggaaagatcgccgtgtaagccataccacatttgtagaggttttacttgctttaaaaaacctcccacacctccccctgaacctgaaacataaaatgaatgcaattgttgttgttaacttgtttattgcagcttataatggttacaaataaagcaatagcatcacaaatttcacaaataaagcatttttttcactgcattctagttgtggtttgtccgaaaggacaaaccataatcgcgtggatatggcacgcaagtttctaccgggcaccgtaaatgtccgactggtttgtaaactcatcaatgtatcttaacgcgt

SEQ ID NO: 6 - DNA, 332 bp, Artificial Sequence
  Synthetic construct
aaggccaagaagggcggaaagatcgccgtgtaagccataccacatttgtagaggttttacttgctttaaaaaacctcccacacctccccctgaacctgaaacataaaatgaatgcaattgttgttgttaacttgtttattgcagcttataatggttacaaataaagcaatagcatcacaaatttcacaaataaagcatttttttcactgcattctagttgtggtttgtccgaaaggacaaaccaataatcgcgtggatatggcacgcaagtttctaccgggcaccgtaaatgtccgacttggtttgaaactcatcaatgtatcttaacgcgt

SEQ ID NO: 7 - DNA, 335 bp, Artificial Sequence
  Synthetic construct
aaggccaagaagggcggaaagatcgccgtgtaagccataccacatttgtagaggttttacttgctttaaaaaacctcccacacctccccctgaacctgaaacataaaatgaatgcaattgttgttgttaacttgtttattgcagcttataatggttacaaataaagcaatagcatcacaaatttcacaaataaagcatttttttcactgcattctagttgtggtttgtccgaaaggacaaaccacaataatcgcgtggatatggcacgcaagtttctaccgggcaccgtaaatgtccgacttgtggtttaaactcatcaatgtatcttaacgcgt

SEQ ID NO: 8 - DNA, 336 bp, Artificial Sequence
  Synthetic construct
aaggccaagaagggcggaaagatcgccgtgtaagccataccacatttgtagaggttttacttgctttaaaaaacctcccacacctccccctgaacctgaaacataaaatgaatgcaattgttgttgttaacttgtttattgcagcttataatggttacaaataaagcaatagcatcacaaatttcacaaataaagcatttttttcactgcattctagttgtggtttgtccgaaaggacaaaccacaacataatcgcgtggatatggcacgcaagtttctaccgggcaccgtaaatgtccgactgttgtggaaactcatcaatgtatcttaacgcgt

SEQ ID NO: 9 - DNA, 158 bp, Artificial Sequence
  Synthetic construct
aaggccaagaagggcggaaagatcgccgtgtaaggatccaagcttatcgataccgtcgacctcgagggcccagatctgcggccgcaataaaagatctttattttcattagatctgtgtgttggttttttgtgtgtctagaaataattcttactgtcat

SEQ ID NO: 10 - DNA, 228 bp, Artificial Sequence
  Synthetic construct
aaggccaagaagggcggaaagatcgccgtgtaaggatccaagcttatcgataccgtcgacctcgagggcccagatctgcggcaaaaggtataatcgcgtggatatggcacgcaagtttctaccgggcaccgtaaatgtccgactaccttttattggaaacaataaaagatctttattttcattagatctgtgtgttggttttttgtgtgtctagaaataattcttact

SEQ ID NO: 11 - DNA, 228 bp, Artificial Sequence
  Synthetic construct
aaggccaagaagggcggaaagatcgccgtgtaaggatccaagcttatcgataccgtcgacctcgagggcccagatctgcggccgcaataaaagatctttattttcattagatctgtgtgttggttttttgtgtgtcgaaagacacacaatataatcgcgtggatatggcacgcaagtttctaccgggcaccgtaaatgtccgactattgtgtggaaataattcttact

SEQ ID NO: 12 - DNA, 153 bp, Artificial Sequence
  Synthetic construct
aaggccaagaagggcggaaagatcgccgtgtaaggatccaagcttatcgataccgtcgacctcgagggcccagatctgcggccgcaataaaatatctttattttcattacatctgtgtgttggttttttgtgtgtctagaaataattcttact

SEQ ID NO: 13 - DNA, 229 bp, Artificial Sequence
  Synthetic construct
aaggccaagaagggcggaaagatcgccgtgtaaggatccaagcttatcgataccgtcgacctcgagggcccagatctgcggaaaaggtataatcgcgtggatatggcacgcaagtttctaccgggcaccgtaaatgtccgactaccttttattgcgaaagcaataaaatatctttattttcattacatctgtgtgttggttttttgtgtgtctagaaataattcttact

SEQ ID NO: 14 - DNA, 332 bp, Artificial Sequence
  Synthetic construct
aaggccaagaagggcggaaagatcgccgtgtaagccataccacatttgtagaggttttacttgctttaaaaaacctcccacacctccccctgaacctgaaacataaaatgaatgcaattgttgttgttaacttgtttattgcagcttataatggttacaaataaagcaatagcatcacaaatttctaaaggtataatcgcgtggatatggcacgcaagtttctaccgggcaccgtaaatgtccgactacctttatttcttcggaaataaagcatttttttcactgcattctagttgtggtttgtccaaactcatcaatgtatcttaacgcgt

SEQ ID NO: 15 - DNA, 332 bp, Artificial Sequence
  Synthetic construct
aaggccaagaagggcggaaagatcgccgtgtaagccataccacatttgtagaggttttacttgctttaaaaaacctcccacacctccccctgaacctgaaacataaaatgaatgcaattgttgttgttaacttgtttattgcagcttataatggttacaaataaagcaatagcatcacaaatttctaaaggtataatcgcgtggatatggcacgcaagtttctaccgggcaccgtaaatgtccgactacctttatttcgaatgaaataaagcatttttttcactgcattctagttgtggtttgtccaaactcatcaatgtatcttaacgcgt

SEQ ID NO: 16 - DNA, 407 bp, Artificial Sequence
  Synthetic construct
aaggccaagaagggcggaaagatcgccgtgtaagccataccacatttgtagaggttttacttgctttaaaaaacctcccacacctccccctgaacctgaaacataaaatgaatgcaattgttgttgttaacttgtttattgcagcttataatggttacaaataaagcaatagcatcacaaatttctaaaggtataatcgcgtggatatggcacgcaagtttctaccgggcaccgtaaatgtccgactacctttatttcgaaagaaataaagcatttttttcactgcattctagttgtggtttgtccgaaaggacaaaccataatcgcgtggatatggcacgcaagtttctaccgggcaccgtaaatgtccgactggtttgtaaactcatcaatgtatcttaacgcgt

SEQ ID NO: 17 - DNA, 334 bp, Artificial Sequence
  Synthetic construct
aaggccaagaagggcggaaagatcgccgtgtaagccataccacatttgtagaggttttacttgctttaaaaaacctcccacacctccccctgaacctgaaacataaaatgaatgcaattgttgttgttaacttgtttattgcagcttataatggttacaaataaagcaatagcatcacaaatttcaataaaggtataacctcaataatatggtttgagggtgtctaccaggaaccgtaaaatcctgattacctttatttcttcggaaataaagcatttttttcactgcattctagttgtggtttgtccaaactcatcaatgtatcttaacgcgt